European Patent Specification EP 3 498 864 B1, published October 9, 2024. Title: METHODS AND COMPOSITIONS FOR THE SELECTION AND OPTIMIZATION OF OLIGONUCLEOTIDE TAG SEQUENCES. Applicant: Gen-Probe Incorporated Nelson, Norman Chelliserry, Jijumon. The sequence listing filed with the application follows.

SEQUENCE LISTING (409 sequences)

SEQ ID NO: 1 - DNA, 20 bp, Artificial Sequence
  Synthetic Oligonucleotide Sequence
gtcatatgcgacgatctcag

SEQ ID NO: 2 - DNA, 30 bp, Artificial Sequence
  Synthetic Oligonucleotide Sequence
ccccgtcaaacaaaaacgggagcgtgtacc

SEQ ID NO: 3 - DNA, 30 bp, Artificial Sequence
  Synthetic Oligonucleotide Sequence
ccataggccttctgcactgctccatatacc

SEQ ID NO: 4 - DNA, 30 bp, Artificial Sequence
  Synthetic Oligonucleotide Sequence
gtccccatcggagggcatcttatcgtgcct

SEQ ID NO: 5 - DNA, 30 bp, Artificial Sequence
  Synthetic Oligonucleotide Sequence
ccgccctccttcgccccccggtgaaataac

SEQ ID NO: 6 - DNA, 30 bp, Artificial Sequence
  Synthetic Oligonucleotide Sequence
aatgctcacctctattcgggacttgagtac

SEQ ID NO: 7 - DNA, 30 bp, Artificial Sequence
  Synthetic Oligonucleotide Sequence
cccgcgcaccacctccatcacgcagaagag

SEQ ID NO: 8 - DNA, 30 bp, Artificial Sequence
  Synthetic Oligonucleotide Sequence
gtcggaacgccaggtacagttagcgcatcc

SEQ ID NO: 9 - DNA, 30 bp, Artificial Sequence
  Synthetic Oligonucleotide Sequence
aagtcactggccagcataatgcgtgaaggg

SEQ ID NO: 10 - DNA, 30 bp, Artificial Sequence
  Synthetic Oligonucleotide Sequence
gtgatgctttatgagattccggtctccgac

SEQ ID NO: 11 - DNA, 30 bp, Artificial Sequence
  Synthetic Oligonucleotide Sequence
gacggtgcatcacccgcatttgctgtagcg

SEQ ID NO: 12 - DNA, 30 bp, Artificial Sequence
  Synthetic Oligonucleotide Sequence
agaattcttgcaggtagaggtcccctcatt

SEQ ID NO: 13 - DNA, 30 bp, Artificial Sequence
  Synthetic Oligonucleotide Sequence
aagccaaaattacaatcgatccctaccaac

SEQ ID NO: 14 - DNA, 30 bp, Artificial Sequence
  Synthetic Oligonucleotide Sequence
atcttgcaccttcccagatgtaaaccccct

SEQ ID NO: 15 - DNA, 30 bp, Artificial Sequence
  Synthetic Oligonucleotide Sequence
gaagcggcagctcagccggttctcggagag

SEQ ID NO: 16 - DNA, 30 bp, Artificial Sequence
  Synthetic Oligonucleotide Sequence
gcacgcgggctccttgggacactatgattg

SEQ ID NO: 17 - DNA, 30 bp, Artificial Sequence
  Synthetic Oligonucleotide Sequence
cccatcaggacagtcagctgcccacgaatt

SEQ ID NO: 18 - DNA, 30 bp, Artificial Sequence
  Synthetic Oligonucleotide Sequence
ctttagtgcggtaggaccgagactaccgtg

SEQ ID NO: 19 - DNA, 30 bp, Artificial Sequence
  Synthetic Oligonucleotide Sequence
ttatgtgccagctgggcctaaggctccggg

SEQ ID NO: 20 - DNA, 30 bp, Artificial Sequence
  Synthetic Oligonucleotide Sequence
gactctcctagggcgttcgtctgggactgc

SEQ ID NO: 21 - DNA, 30 bp, Artificial Sequence
  Synthetic Oligonucleotide Sequence
cggagaataccctcgactgtatcatatcgt

SEQ ID NO: 22 - DNA, 30 bp, Artificial Sequence
  Synthetic Oligonucleotide Sequence
ttcatcgaggtacattggtgctattccatt

SEQ ID NO: 23 - DNA, 30 bp, Artificial Sequence
  Synthetic Oligonucleotide Sequence
taccacctggttcaaggtgtgccgtacgcg

SEQ ID NO: 24 - DNA, 30 bp, Artificial Sequence
  Synthetic Oligonucleotide Sequence
aggagaaccagcctggagcgtttaagcatc

SEQ ID NO: 25 - DNA, 30 bp, Artificial Sequence
  Synthetic Oligonucleotide Sequence
gatgtcctaaaatgaggcgtggcaatagag

SEQ ID NO: 26 - DNA, 30 bp, Artificial Sequence
  Synthetic Oligonucleotide Sequence
cagagtcatgtatacccactgtcggtcgaa

SEQ ID NO: 27 - DNA, 30 bp, Artificial Sequence
  Synthetic Oligonucleotide Sequence
gtcaggctagggggttatcccagcaacggc

SEQ ID NO: 28 - DNA, 30 bp, Artificial Sequence
  Synthetic Oligonucleotide Sequence
tgggttctgctaaccggtgccgttcttaac

SEQ ID NO: 29 - DNA, 30 bp, Artificial Sequence
  Synthetic Oligonucleotide Sequence
tttttgacagtgatgaagagggaggtacga

SEQ ID NO: 30 - DNA, 30 bp, Artificial Sequence
  Synthetic Oligonucleotide Sequence
gagaactcgcgctccctcactccgtttaga

SEQ ID NO: 31 - DNA, 30 bp, Artificial Sequence
  Synthetic Oligonucleotide Sequence
ctatggttcgttactgaatcgaaaagccgc

SEQ ID NO: 32 - DNA, 30 bp, Artificial Sequence
  Synthetic Oligonucleotide Sequence
tagctatcaaaacaggcgtcatcggttaag

SEQ ID NO: 33 - DNA, 30 bp, Artificial Sequence
  Synthetic Oligonucleotide Sequence
aggacgctgacaccgttggggtaaagcgtg

SEQ ID NO: 34 - DNA, 30 bp, Artificial Sequence
  Synthetic Oligonucleotide Sequence
cctgcttagggtcacttaaactactggcgc

SEQ ID NO: 35 - DNA, 30 bp, Artificial Sequence
  Synthetic Oligonucleotide Sequence
ggtgatggcccataccgatcacgcccgcag

SEQ ID NO: 36 - DNA, 30 bp, Artificial Sequence
  Synthetic Oligonucleotide Sequence
cggcaggagggactgcgatttccatagagc

SEQ ID NO: 37 - DNA, 30 bp, Artificial Sequence
  Synthetic Oligonucleotide Sequence
tggccggagagaggataggaagcgggacta

SEQ ID NO: 38 - DNA, 30 bp, Artificial Sequence
  Synthetic Oligonucleotide Sequence
tagcaggtgtctcggtcctcaactgcaaac

SEQ ID NO: 39 - DNA, 30 bp, Artificial Sequence
  Synthetic Oligonucleotide Sequence
acacatcccaggactgccgtggcctacgta

SEQ ID NO: 40 - DNA, 30 bp, Artificial Sequence
  Synthetic Oligonucleotide Sequence
gtgctagcccgggcccttcttaactcggga

SEQ ID NO: 41 - DNA, 30 bp, Artificial Sequence
  Synthetic Oligonucleotide Sequence
cggaatctgaacatctatcagagccgcgct

SEQ ID NO: 42 - DNA, 30 bp, Artificial Sequence
  Synthetic Oligonucleotide Sequence
gacgagcttgttccaattcctcgagccgag

SEQ ID NO: 43 - DNA, 30 bp, Artificial Sequence
  Synthetic Oligonucleotide Sequence
gttggggaggggcactacgacttagggcta

SEQ ID NO: 44 - DNA, 30 bp, Artificial Sequence
  Synthetic Oligonucleotide Sequence
aatgtggacggccgctccgtacttctgaca

SEQ ID NO: 45 - DNA, 30 bp, Artificial Sequence
  Synthetic Oligonucleotide Sequence
agggccagcagctggttccttcgccagtta

SEQ ID NO: 46 - DNA, 30 bp, Artificial Sequence
  Synthetic Oligonucleotide Sequence
ggccgtcaatgtgttttgcacccaaccgga

SEQ ID NO: 47 - DNA, 30 bp, Artificial Sequence
  Synthetic Oligonucleotide Sequence
cagtgactgggctagtgaagtgagtcacag

SEQ ID NO: 48 - DNA, 30 bp, Artificial Sequence
  Synthetic Oligonucleotide Sequence
tcccacgtccttcgacgcacactgtaactt

SEQ ID NO: 49 - DNA, 25 bp, Artificial Sequence
  Synthetic Oligonucleotide Sequence
tcatgtatcgcccgtgggtaagctc

SEQ ID NO: 50 - DNA, 25 bp, Artificial Sequence
  Synthetic Oligonucleotide Sequence
atgttatggagagtgggttaggcaa

SEQ ID NO: 51 - DNA, 25 bp, Artificial Sequence
  Synthetic Oligonucleotide Sequence
atgagggagtaaggagattaggttc

SEQ ID NO: 52 - DNA, 25 bp, Artificial Sequence
  Synthetic Oligonucleotide Sequence
catgctgcccgcatacacttgcggg

SEQ ID NO: 53 - DNA, 25 bp, Artificial Sequence
  Synthetic Oligonucleotide Sequence
gcccagcagttatacaattcgtggc

SEQ ID NO: 54 - DNA, 25 bp, Artificial Sequence
  Synthetic Oligonucleotide Sequence
ttgggctctccagtagccgaacaaa

SEQ ID NO: 55 - DNA, 25 bp, Artificial Sequence
  Synthetic Oligonucleotide Sequence
tgacgttaaacgcaatccgcgtaaa

SEQ ID NO: 56 - DNA, 25 bp, Artificial Sequence
  Synthetic Oligonucleotide Sequence
gtcgccattcaggacacgcgaaact

SEQ ID NO: 57 - DNA, 25 bp, Artificial Sequence
  Synthetic Oligonucleotide Sequence
gtggttgctacagcctagcctagat

SEQ ID NO: 58 - DNA, 25 bp, Artificial Sequence
  Synthetic Oligonucleotide Sequence
ccacttttcattccgagtccacgcg

SEQ ID NO: 59 - DNA, 25 bp, Artificial Sequence
  Synthetic Oligonucleotide Sequence
aggaggaaccggaagatctaatctg

SEQ ID NO: 60 - DNA, 25 bp, Artificial Sequence
  Synthetic Oligonucleotide Sequence
ccaatgctttcaaataacccgttct

SEQ ID NO: 61 - DNA, 25 bp, Artificial Sequence
  Synthetic Oligonucleotide Sequence
gcgactgtggcaaccccatttcgca

SEQ ID NO: 62 - DNA, 25 bp, Artificial Sequence
  Synthetic Oligonucleotide Sequence
aaaaaacggaggagtcgaaccttgg

SEQ ID NO: 63 - DNA, 25 bp, Artificial Sequence
  Synthetic Oligonucleotide Sequence
agttggatggatatctcgctcgtga

SEQ ID NO: 64 - DNA, 25 bp, Artificial Sequence
  Synthetic Oligonucleotide Sequence
cgctgtcctctctgacactaaaggt

SEQ ID NO: 65 - DNA, 25 bp, Artificial Sequence
  Synthetic Oligonucleotide Sequence
atttcaatagtcaacccggtatcca

SEQ ID NO: 66 - DNA, 25 bp, Artificial Sequence
  Synthetic Oligonucleotide Sequence
ttcgcgccagcgaccccacttatga

SEQ ID NO: 67 - DNA, 25 bp, Artificial Sequence
  Synthetic Oligonucleotide Sequence
ggttggggggctcggctcatgtatc

SEQ ID NO: 68 - DNA, 25 bp, Artificial Sequence
  Synthetic Oligonucleotide Sequence
atgatgctgaatcgcgatggggggg

SEQ ID NO: 69 - DNA, 25 bp, Artificial Sequence
  Synthetic Oligonucleotide Sequence
taaggagactaggttccaatagctg

SEQ ID NO: 70 - DNA, 25 bp, Artificial Sequence
  Synthetic Oligonucleotide Sequence
ttacacaaatcgtgggttggcctct

SEQ ID NO: 71 - DNA, 25 bp, Artificial Sequence
  Synthetic Oligonucleotide Sequence
cgaaagcgttccgcaggaccccctt

SEQ ID NO: 72 - DNA, 25 bp, Artificial Sequence
  Synthetic Oligonucleotide Sequence
cacccttggacacgtggaagtgggc

SEQ ID NO: 73 - DNA, 25 bp, Artificial Sequence
  Synthetic Oligonucleotide Sequence
aaagtctgagaatgagtgataccat

SEQ ID NO: 74 - DNA, 25 bp, Artificial Sequence
  Synthetic Oligonucleotide Sequence
atattggtagttttgtccgctgtag

SEQ ID NO: 75 - DNA, 25 bp, Artificial Sequence
  Synthetic Oligonucleotide Sequence
cggaagatctaatctgcacgcaatt

SEQ ID NO: 76 - DNA, 30 bp, Artificial Sequence
  Synthetic Oligonucleotide Sequence
gcgcctcgttgggcagaagtttgtggaaat

SEQ ID NO: 77 - DNA, 30 bp, Artificial Sequence
  Synthetic Oligonucleotide Sequence
atcttcacctaccgagttctacgggcctac

SEQ ID NO: 78 - DNA, 30 bp, Artificial Sequence
  Synthetic Oligonucleotide Sequence
cccacaacttgcacccgctatgcgaccctg

SEQ ID NO: 79 - DNA, 30 bp, Artificial Sequence
  Synthetic Oligonucleotide Sequence
gcccaggagctctcctgggtaacagtagcg

SEQ ID NO: 80 - DNA, 30 bp, Artificial Sequence
  Synthetic Oligonucleotide Sequence
cacggcccccaggcggcgtatcagggatga

SEQ ID NO: 81 - DNA, 30 bp, Artificial Sequence
  Synthetic Oligonucleotide Sequence
tccccggcacggaccgcaagggaccaaagc

SEQ ID NO: 82 - DNA, 30 bp, Artificial Sequence
  Synthetic Oligonucleotide Sequence
gattagtggcccaacgggaacaaacttcct

SEQ ID NO: 83 - DNA, 30 bp, Artificial Sequence
  Synthetic Oligonucleotide Sequence
cgcccgtcccagacccttactcactatgga

SEQ ID NO: 84 - DNA, 30 bp, Artificial Sequence
  Synthetic Oligonucleotide Sequence
gctacacgccagaggcgccgctacagcgat

SEQ ID NO: 85 - DNA, 30 bp, Artificial Sequence
  Synthetic Oligonucleotide Sequence
gagattgtaccctacagtccgattaccgat

SEQ ID NO: 86 - DNA, 30 bp, Artificial Sequence
  Synthetic Oligonucleotide Sequence
cgcagtaaaagggcacaggtaattacctta

SEQ ID NO: 87 - DNA, 30 bp, Artificial Sequence
  Synthetic Oligonucleotide Sequence
agggtgtcttgaactactggcgcagcccat

SEQ ID NO: 88 - DNA, 30 bp, Artificial Sequence
  Synthetic Oligonucleotide Sequence
ccgcaatccggtgacggccggaccggcagg

SEQ ID NO: 89 - DNA, 30 bp, Artificial Sequence
  Synthetic Oligonucleotide Sequence
tcggcggcgggtagtcagttcgctacctgg

SEQ ID NO: 90 - DNA, 30 bp, Artificial Sequence
  Synthetic Oligonucleotide Sequence
ccaggactgccgtggcccacgcactcacga

SEQ ID NO: 91 - DNA, 30 bp, Artificial Sequence
  Synthetic Oligonucleotide Sequence
ttgacgcaggcccccggggcgacttcatac

SEQ ID NO: 92 - DNA, 30 bp, Artificial Sequence
  Synthetic Oligonucleotide Sequence
cgaaaggagttcgagtgtatccggaaggcg

SEQ ID NO: 93 - DNA, 30 bp, Artificial Sequence
  Synthetic Oligonucleotide Sequence
aggcgcactgcgacttagggctagcccccc

SEQ ID NO: 94 - DNA, 30 bp, Artificial Sequence
  Synthetic Oligonucleotide Sequence
gatgtgatctggaccctacgggaggggaca

SEQ ID NO: 95 - DNA, 30 bp, Artificial Sequence
  Synthetic Oligonucleotide Sequence
tgggctgggggagtgagtcgctcccgcagc

SEQ ID NO: 96 - DNA, 30 bp, Artificial Sequence
  Synthetic Oligonucleotide Sequence
agtcccagatatgagagaagcgaagcataa

SEQ ID NO: 97 - DNA, 25 bp, Artificial Sequence
  Synthetic Oligonucleotide Sequence
cgtttcagcatcgatgtcctaaaat

SEQ ID NO: 98 - DNA, 25 bp, Artificial Sequence
  Synthetic Oligonucleotide Sequence
actattacaccacgtaccgtaggtc

SEQ ID NO: 99 - DNA, 25 bp, Artificial Sequence
  Synthetic Oligonucleotide Sequence
gggcaacaccgcgagctaattatcc

SEQ ID NO: 100 - DNA, 25 bp, Artificial Sequence
  Synthetic Oligonucleotide Sequence
gcgcgcggccgagaatcgttggagg

SEQ ID NO: 101 - DNA, 25 bp, Artificial Sequence
  Synthetic Oligonucleotide Sequence
cgcgtcgggctttcgtctaccctgg

SEQ ID NO: 102 - DNA, 25 bp, Artificial Sequence
  Synthetic Oligonucleotide Sequence
gggcggccaccgggggaccctgccc

SEQ ID NO: 103 - DNA, 12 bp, Artificial Sequence
  Synthetic Oligonucleotide Sequence
tggctaatcccg

SEQ ID NO: 104 - DNA, 16 bp, Artificial Sequence
  Synthetic Oligonucleotide Sequence
gcgttggctaatcccg

SEQ ID NO: 105 - DNA, 12 bp, Artificial Sequence
  Synthetic Oligonucleotide Sequence
ctgtgctagagg

SEQ ID NO: 106 - DNA, 12 bp, Artificial Sequence
  Synthetic Oligonucleotide Sequence
catgtaccaacg

SEQ ID NO: 107 - DNA, 16 bp, Artificial Sequence
  Synthetic Oligonucleotide Sequence
tcaccatgtaccaacg

SEQ ID NO: 108 - DNA, 12 bp, Artificial Sequence
  Synthetic Oligonucleotide Sequence
tcggtcggacta

SEQ ID NO: 109 - DNA, 12 bp, Artificial Sequence
  Synthetic Oligonucleotide Sequence
cctcccccaagc

SEQ ID NO: 110 - DNA, 12 bp, Artificial Sequence
  Synthetic Oligonucleotide Sequence
gggtttgctacg

SEQ ID NO: 111 - DNA, 12 bp, Artificial Sequence
  Synthetic Oligonucleotide Sequence
atgtgcgcacaa

SEQ ID NO: 112 - DNA, 12 bp, Artificial Sequence
  Synthetic Oligonucleotide Sequence
cgggactagaga

SEQ ID NO: 113 - DNA, 12 bp, Artificial Sequence
  Synthetic Oligonucleotide Sequence
aatctccgagcg

SEQ ID NO: 114 - DNA, 12 bp, Artificial Sequence
  Synthetic Oligonucleotide Sequence
aagtgcaggttc

SEQ ID NO: 115 - DNA, 12 bp, Artificial Sequence
  Synthetic Oligonucleotide Sequence
tccagtttaacc

SEQ ID NO: 116 - DNA, 12 bp, Artificial Sequence
  Synthetic Oligonucleotide Sequence
tagccgcacagg

SEQ ID NO: 117 - DNA, 18 bp, Artificial Sequence
  Synthetic Oligonucleotide Sequence
tatgaatgcgacccggaa

SEQ ID NO: 118 - DNA, 18 bp, Artificial Sequence
  Synthetic Oligonucleotide Sequence
aacaatggtcactgcatc

SEQ ID NO: 119 - DNA, 20 bp, Artificial Sequence
  Synthetic Oligonucleotide Sequence
gggccgtttcccggacataa

SEQ ID NO: 120 - DNA, 20 bp, Artificial Sequence
  Synthetic Oligonucleotide Sequence
aggttgagtccgcatctgaa

SEQ ID NO: 121 - DNA, 22 bp, Artificial Sequence
  Synthetic Oligonucleotide Sequence
tcgaccaagagccgctagatgc

SEQ ID NO: 122 - DNA, 22 bp, Artificial Sequence
  Synthetic Oligonucleotide Sequence
agctcgtgtcaagccgtcgcct

SEQ ID NO: 123 - DNA, 24 bp, Artificial Sequence
  Synthetic Oligonucleotide Sequence
tgaaagagttgtcagtttgctggt

SEQ ID NO: 124 - DNA, 25 bp, Artificial Sequence
  Synthetic Oligonucleotide Sequence
tcaggtaaaggttcctcacgctacc

SEQ ID NO: 125 - DNA, 25 bp, Artificial Sequence
  Synthetic Oligonucleotide Sequence
cccataacttggtgcgaatacgggt

SEQ ID NO: 126 - DNA, 25 bp, Artificial Sequence
  Synthetic Oligonucleotide Sequence
cgtagcaatgttcgtctgactatga

SEQ ID NO: 127 - DNA, 25 bp, Artificial Sequence
  Synthetic Oligonucleotide Sequence
caactacggggattcttggagagcc

SEQ ID NO: 128 - DNA, 25 bp, Artificial Sequence
  Synthetic Oligonucleotide Sequence
gtgtagtattagcaaacgataagtc

SEQ ID NO: 129 - DNA, 25 bp, Artificial Sequence
  Synthetic Oligonucleotide Sequence
cgggggctgggaatctgtgacatga

SEQ ID NO: 130 - DNA, 25 bp, Artificial Sequence
  Synthetic Oligonucleotide Sequence
tgcctgtcgatccataggactcgtg

SEQ ID NO: 131 - DNA, 25 bp, Artificial Sequence
  Synthetic Oligonucleotide Sequence
gaaatgtccggggccaaagacaacc

SEQ ID NO: 132 - DNA, 25 bp, Artificial Sequence
  Synthetic Oligonucleotide Sequence
ctgacatagtatagcatagatattg

SEQ ID NO: 133 - DNA, 25 bp, Artificial Sequence
  Synthetic Oligonucleotide Sequence
gaatttatagatactgccaatctag

SEQ ID NO: 134 - DNA, 25 bp, Artificial Sequence
  Synthetic Oligonucleotide Sequence
atcagttggacagagggctgtgtta

SEQ ID NO: 135 - DNA, 25 bp, Artificial Sequence
  Synthetic Oligonucleotide Sequence
cttctagagaagaagagtactgact

SEQ ID NO: 136 - DNA, 25 bp, Artificial Sequence
  Synthetic Oligonucleotide Sequence
ggttcagttgtaaccatatacttac

SEQ ID NO: 137 - DNA, 25 bp, Artificial Sequence
  Synthetic Oligonucleotide Sequence
aatgacgtagctatgtattttgcac

SEQ ID NO: 138 - DNA, 25 bp, Artificial Sequence
  Synthetic Oligonucleotide Sequence
aggtagccaacgggtttcacatttc

SEQ ID NO: 139 - DNA, 25 bp, Artificial Sequence
  Synthetic Oligonucleotide Sequence
gcgtaaactacgatggcacctactc

SEQ ID NO: 140 - DNA, 25 bp, Artificial Sequence
  Synthetic Oligonucleotide Sequence
ctcataacttggtgcgaatacgggt

SEQ ID NO: 141 - DNA, 25 bp, Artificial Sequence
  Synthetic Oligonucleotide Sequence
tgtagcaatgttcgtctgactatga

SEQ ID NO: 142 - DNA, 25 bp, Artificial Sequence
  Synthetic Oligonucleotide Sequence
taaaatagtacagctactggtgatc

SEQ ID NO: 143 - DNA, 25 bp, Artificial Sequence
  Synthetic Oligonucleotide Sequence
caactacgaggatttttagagagcc

SEQ ID NO: 144 - DNA, 25 bp, Artificial Sequence
  Synthetic Oligonucleotide Sequence
atgtagtattagcaaacaataagtc

SEQ ID NO: 145 - DNA, 25 bp, Artificial Sequence
  Synthetic Oligonucleotide Sequence
aattgaatggagtctgatcaatctt

SEQ ID NO: 146 - DNA, 25 bp, Artificial Sequence
  Synthetic Oligonucleotide Sequence
gaagttggaggattaacgtgggaat

SEQ ID NO: 147 - DNA, 25 bp, Artificial Sequence
  Synthetic Oligonucleotide Sequence
ggtttactattgtctctaatgggag

SEQ ID NO: 148 - DNA, 25 bp, Artificial Sequence
  Synthetic Oligonucleotide Sequence
ttgacatagtatagcatagatattg

SEQ ID NO: 149 - DNA, 25 bp, Artificial Sequence
  Synthetic Oligonucleotide Sequence
cagataacttacctacattgaaagt

SEQ ID NO: 150 - DNA, 25 bp, Artificial Sequence
  Synthetic Oligonucleotide Sequence
tatagacgactattccgactagcaa

SEQ ID NO: 151 - DNA, 25 bp, Artificial Sequence
  Synthetic Oligonucleotide Sequence
gaatttatagatactaccaatctag

SEQ ID NO: 152 - DNA, 25 bp, Artificial Sequence
  Synthetic Oligonucleotide Sequence
attaattggacagagggctgtgtta

SEQ ID NO: 153 - DNA, 25 bp, Artificial Sequence
  Synthetic Oligonucleotide Sequence
ctgttgccactctttagaaagatta

SEQ ID NO: 154 - DNA, 25 bp, Artificial Sequence
  Synthetic Oligonucleotide Sequence
actacaataataccaactatttgcc

SEQ ID NO: 155 - DNA, 25 bp, Artificial Sequence
  Synthetic Oligonucleotide Sequence
gatactaaataacaacttagttttt

SEQ ID NO: 156 - DNA, 25 bp, Artificial Sequence
  Synthetic Oligonucleotide Sequence
tagatttcattccgagtccacatgt

SEQ ID NO: 157 - DNA, 25 bp, Artificial Sequence
  Synthetic Oligonucleotide Sequence
aactctaatataagatatcaagtta

SEQ ID NO: 158 - DNA, 25 bp, Artificial Sequence
  Synthetic Oligonucleotide Sequence
attgttaaagtagactaattatcta

SEQ ID NO: 159 - DNA, 25 bp, Artificial Sequence
  Synthetic Oligonucleotide Sequence
gaaggaactggaagatttaatttgc

SEQ ID NO: 160 - DNA, 25 bp, Artificial Sequence
  Synthetic Oligonucleotide Sequence
acgcaattaatatacatatttatac

SEQ ID NO: 161 - DNA, 25 bp, Artificial Sequence
  Synthetic Oligonucleotide Sequence
caattatgcgaattccatttcacat

SEQ ID NO: 162 - DNA, 25 bp, Artificial Sequence
  Synthetic Oligonucleotide Sequence
cttatgagatgttagatatagtatt

SEQ ID NO: 163 - DNA, 25 bp, Artificial Sequence
  Synthetic Oligonucleotide Sequence
cttttacaatatcagactttagcaa

SEQ ID NO: 164 - DNA, 25 bp, Artificial Sequence
  Synthetic Oligonucleotide Sequence
gatgtagacggattccatagaattt

SEQ ID NO: 165 - DNA, 25 bp, Artificial Sequence
  Synthetic Oligonucleotide Sequence
aatgattgtgtggagtacaaaccaa

SEQ ID NO: 166 - DNA, 25 bp, Artificial Sequence
  Synthetic Oligonucleotide Sequence
tttttttggcgtaaagtctagagtt

SEQ ID NO: 167 - DNA, 25 bp, Artificial Sequence
  Synthetic Oligonucleotide Sequence
atcacgtaagaccactgttagtata

SEQ ID NO: 168 - DNA, 25 bp, Artificial Sequence
  Synthetic Oligonucleotide Sequence
ctttaatagtcaaaccgatatccat

SEQ ID NO: 169 - DNA, 25 bp, Artificial Sequence
  Synthetic Oligonucleotide Sequence
cagtcaagtgatggactctaacaca

SEQ ID NO: 170 - DNA, 25 bp, Artificial Sequence
  Synthetic Oligonucleotide Sequence
tcattagcggaaaaaactgaccttc

SEQ ID NO: 171 - DNA, 25 bp, Artificial Sequence
  Synthetic Oligonucleotide Sequence
ctcctatccttcgccacaactttag

SEQ ID NO: 172 - DNA, 25 bp, Artificial Sequence
  Synthetic Oligonucleotide Sequence
ttgctttgagattgaaatataaaag

SEQ ID NO: 173 - DNA, 25 bp, Artificial Sequence
  Synthetic Oligonucleotide Sequence
atcatatacagtgccagggaacaac

SEQ ID NO: 174 - DNA, 25 bp, Artificial Sequence
  Synthetic Oligonucleotide Sequence
acttgtagaaataccttataaagtt

SEQ ID NO: 175 - DNA, 25 bp, Artificial Sequence
  Synthetic Oligonucleotide Sequence
attcttgatgtatgtagagtcctaa

SEQ ID NO: 176 - DNA, 25 bp, Artificial Sequence
  Synthetic Oligonucleotide Sequence
tgatatcgaatacataagtactcga

SEQ ID NO: 177 - DNA, 25 bp, Artificial Sequence
  Synthetic Oligonucleotide Sequence
atgactgaattgcttacacatttaa

SEQ ID NO: 178 - DNA, 25 bp, Artificial Sequence
  Synthetic Oligonucleotide Sequence
aaaaacaattagtatataactatta

SEQ ID NO: 179 - DNA, 25 bp, Artificial Sequence
  Synthetic Oligonucleotide Sequence
taatagtgtcatcggctccacttat

SEQ ID NO: 180 - DNA, 25 bp, Artificial Sequence
  Synthetic Oligonucleotide Sequence
tacaatcaaaacgtgaagttattga

SEQ ID NO: 181 - DNA, 25 bp, Artificial Sequence
  Synthetic Oligonucleotide Sequence
gtttagttattgacttgtagatagt

SEQ ID NO: 182 - DNA, 25 bp, Artificial Sequence
  Synthetic Oligonucleotide Sequence
ctcgacaccgagtgctagatcaacg

SEQ ID NO: 183 - DNA, 25 bp, Artificial Sequence
  Synthetic Oligonucleotide Sequence
acccggacatattggctattcaaac

SEQ ID NO: 184 - DNA, 25 bp, Artificial Sequence
  Synthetic Oligonucleotide Sequence
aatatttaaaagcctggtttatgta

SEQ ID NO: 185 - DNA, 25 bp, Artificial Sequence
  Synthetic Oligonucleotide Sequence
ctttagtgccgatttacggccttgg

SEQ ID NO: 186 - DNA, 25 bp, Artificial Sequence
  Synthetic Oligonucleotide Sequence
ggtaagataacgaagttttaatagc

SEQ ID NO: 187 - DNA, 25 bp, Artificial Sequence
  Synthetic Oligonucleotide Sequence
tgctttgacactgttcattataccg

SEQ ID NO: 188 - DNA, 25 bp, Artificial Sequence
  Synthetic Oligonucleotide Sequence
ttttcttttacccactggtgaaata

SEQ ID NO: 189 - DNA, 25 bp, Artificial Sequence
  Synthetic Oligonucleotide Sequence
tcaagattgtccttgattgttgaat

SEQ ID NO: 190 - DNA, 25 bp, Artificial Sequence
  Synthetic Oligonucleotide Sequence
aaagatctgattaacttataacaga

SEQ ID NO: 191 - DNA, 25 bp, Artificial Sequence
  Synthetic Oligonucleotide Sequence
atgaataaatcttgtaaagtgtggc

SEQ ID NO: 192 - DNA, 25 bp, Artificial Sequence
  Synthetic Oligonucleotide Sequence
agctacactaaacctagaatgatct

SEQ ID NO: 193 - DNA, 25 bp, Artificial Sequence
  Synthetic Oligonucleotide Sequence
cttcaatttgagacttgaaatctaa

SEQ ID NO: 194 - DNA, 25 bp, Artificial Sequence
  Synthetic Oligonucleotide Sequence
gtttcactcagtgtagacatcatcc

SEQ ID NO: 195 - DNA, 25 bp, Artificial Sequence
  Synthetic Oligonucleotide Sequence
tggtatctgaattactgctttgtca

SEQ ID NO: 196 - DNA, 25 bp, Artificial Sequence
  Synthetic Oligonucleotide Sequence
aagtgtctattatccttaaacgcat

SEQ ID NO: 197 - DNA, 25 bp, Artificial Sequence
  Synthetic Oligonucleotide Sequence
atctcgcataataactcctcaatat

SEQ ID NO: 198 - DNA, 25 bp, Artificial Sequence
  Synthetic Oligonucleotide Sequence
gagttagtcttgtgctcacggaatt

SEQ ID NO: 199 - DNA, 25 bp, Artificial Sequence
  Synthetic Oligonucleotide Sequence
aaatgttagttagctcgttcaagta

SEQ ID NO: 200 - DNA, 25 bp, Artificial Sequence
  Synthetic Oligonucleotide Sequence
aaagttcttcacactacgtcaaaat

SEQ ID NO: 201 - DNA, 25 bp, Artificial Sequence
  Synthetic Oligonucleotide Sequence
aaaaaaatggttgtaacaaaaaaaa

SEQ ID NO: 202 - DNA, 27 bp, Artificial Sequence
  Synthetic Oligonucleotide Sequence
ggctcatcgatgacccaagatggcggc

SEQ ID NO: 203 - DNA, 27 bp, Artificial Sequence
  Synthetic Oligonucleotide Sequence
tctccctatagtgagtcgtattaaatt

SEQ ID NO: 204 - DNA, 20 bp, Artificial Sequence
  Synthetic Oligonucleotide Sequence
gtctaagtagtgacatgttt

SEQ ID NO: 205 - DNA, 32 bp, Artificial Sequence
  Synthetic Oligonucleotide Sequence
tggctaatcccggtctaagtagtgacatgttt

SEQ ID NO: 206 - DNA, 39 bp, Artificial Sequence
  Synthetic Oligonucleotide Sequence
ggctcatcgatgacccaagatggcggctggctaatcccg

SEQ ID NO: 207 - DNA, 59 bp, Artificial Sequence
  Synthetic Oligonucleotide Sequence
ggctcatcgatgacccaagatggcggctggctaatcccggtctaagtagtgacatgttt

SEQ ID NO: 208 - DNA, 32 bp, Artificial Sequence
  Synthetic Oligonucleotide Sequence
ctgtgctagagggtctaagtagtgacatgttt

SEQ ID NO: 209 - DNA, 39 bp, Artificial Sequence
  Synthetic Oligonucleotide Sequence
ggctcatcgatgacccaagatggcggcctgtgctagagg

SEQ ID NO: 210 - DNA, 59 bp, Artificial Sequence
  Synthetic Oligonucleotide Sequence
ggctcatcgatgacccaagatggcggcctgtgctagagggtctaagtagtgacatgttt

SEQ ID NO: 211 - DNA, 32 bp, Artificial Sequence
  Synthetic Oligonucleotide Sequence
catgtaccaacggtctaagtagtgacatgttt

SEQ ID NO: 212 - DNA, 39 bp, Artificial Sequence
  Synthetic Oligonucleotide Sequence
ggctcatcgatgacccaagatggcggccatgtaccaacg

SEQ ID NO: 213 - DNA, 59 bp, Artificial Sequence
  Synthetic Oligonucleotide Sequence
ggctcatcgatgacccaagatggcggccatgtaccaacggtctaagtagtgacatgttt

SEQ ID NO: 214 - DNA, 32 bp, Artificial Sequence
  Synthetic Oligonucleotide Sequence
tcggtcggactagtctaagtagtgacatgttt

SEQ ID NO: 215 - DNA, 39 bp, Artificial Sequence
  Synthetic Oligonucleotide Sequence
ggctcatcgatgacccaagatggcggctcggtcggacta

SEQ ID NO: 216 - DNA, 59 bp, Artificial Sequence
  Synthetic Oligonucleotide Sequence
ggctcatcgatgacccaagatggcggctcggtcggactagtctaagtagtgacatgttt

SEQ ID NO: 217 - DNA, 32 bp, Artificial Sequence
  Synthetic Oligonucleotide Sequence
cctcccccaagcgtctaagtagtgacatgttt

SEQ ID NO: 218 - DNA, 39 bp, Artificial Sequence
  Synthetic Oligonucleotide Sequence
ggctcatcgatgacccaagatggcggccctcccccaagc

SEQ ID NO: 219 - DNA, 59 bp, Artificial Sequence
  Synthetic Oligonucleotide Sequence
ggctcatcgatgacccaagatggcggccctcccccaagcgtctaagtagtgacatgttt

SEQ ID NO: 220 - DNA, 32 bp, Artificial Sequence
  Synthetic Oligonucleotide Sequence
gggtttgctacggtctaagtagtgacatgttt

SEQ ID NO: 221 - DNA, 39 bp, Artificial Sequence
  Synthetic Oligonucleotide Sequence
ggctcatcgatgacccaagatggcggcgggtttgctacg

SEQ ID NO: 222 - DNA, 59 bp, Artificial Sequence
  Synthetic Oligonucleotide Sequence
ggctcatcgatgacccaagatggcggcgggtttgctacggtctaagtagtgacatgttt

SEQ ID NO: 223 - DNA, 32 bp, Artificial Sequence
  Synthetic Oligonucleotide Sequence
atgtgcgcacaagtctaagtagtgacatgttt

SEQ ID NO: 224 - DNA, 39 bp, Artificial Sequence
  Synthetic Oligonucleotide Sequence
ggctcatcgatgacccaagatggcggcatgtgcgcacaa

SEQ ID NO: 225 - DNA, 59 bp, Artificial Sequence
  Synthetic Oligonucleotide Sequence
ggctcatcgatgacccaagatggcggcatgtgcgcacaagtctaagtagtgacatgttt

SEQ ID NO: 226 - DNA, 32 bp, Artificial Sequence
  Synthetic Oligonucleotide Sequence
cgggactagagagtctaagtagtgacatgttt

SEQ ID NO: 227 - DNA, 39 bp, Artificial Sequence
  Synthetic Oligonucleotide Sequence
ggctcatcgatgacccaagatggcggccgggactagaga

SEQ ID NO: 228 - DNA, 59 bp, Artificial Sequence
  Synthetic Oligonucleotide Sequence
ggctcatcgatgacccaagatggcggccgggactagagagtctaagtagtgacatgttt

SEQ ID NO: 229 - DNA, 32 bp, Artificial Sequence
  Synthetic Oligonucleotide Sequence
aatctccgagcggtctaagtagtgacatgttt

SEQ ID NO: 230 - DNA, 39 bp, Artificial Sequence
  Synthetic Oligonucleotide Sequence
ggctcatcgatgacccaagatggcggcaatctccgagcg

SEQ ID NO: 231 - DNA, 59 bp, Artificial Sequence
  Synthetic Oligonucleotide Sequence
ggctcatcgatgacccaagatggcggcaatctccgagcggtctaagtagtgacatgttt

SEQ ID NO: 232 - DNA, 32 bp, Artificial Sequence
  Synthetic Oligonucleotide Sequence
aagtgcaggttcgtctaagtagtgacatgttt

SEQ ID NO: 233 - DNA, 39 bp, Artificial Sequence
  Synthetic Oligonucleotide Sequence
ggctcatcgatgacccaagatggcggcaagtgcaggttc

SEQ ID NO: 234 - DNA, 59 bp, Artificial Sequence
  Synthetic Oligonucleotide Sequence
ggctcatcgatgacccaagatggcggcaagtgcaggttcgtctaagtagtgacatgttt

SEQ ID NO: 235 - DNA, 32 bp, Artificial Sequence
  Synthetic Oligonucleotide Sequence
tccagtttaaccgtctaagtagtgacatgttt

SEQ ID NO: 236 - DNA, 39 bp, Artificial Sequence
  Synthetic Oligonucleotide Sequence
ggctcatcgatgacccaagatggcggctccagtttaacc

SEQ ID NO: 237 - DNA, 59 bp, Artificial Sequence
  Synthetic Oligonucleotide Sequence
ggctcatcgatgacccaagatggcggctccagtttaaccgtctaagtagtgacatgttt

SEQ ID NO: 238 - DNA, 32 bp, Artificial Sequence
  Synthetic Oligonucleotide Sequence
tagccgcacagggtctaagtagtgacatgttt

SEQ ID NO: 239 - DNA, 39 bp, Artificial Sequence
  Synthetic Oligonucleotide Sequence
ggctcatcgatgacccaagatggcggctagccgcacagg

SEQ ID NO: 240 - DNA, 59 bp, Artificial Sequence
  Synthetic Oligonucleotide Sequence
ggctcatcgatgacccaagatggcggctagccgcacagggtctaagtagtgacatgttt

SEQ ID NO: 241 - DNA, 36 bp, Artificial Sequence
  Synthetic Oligonucleotide Sequence
gcgttggctaatcccggtctaagtagtgacatgttt

SEQ ID NO: 242 - DNA, 43 bp, Artificial Sequence
  Synthetic Oligonucleotide Sequence
ggctcatcgatgacccaagatggcggcgcgttggctaatcccg

SEQ ID NO: 243 - DNA, 63 bp, Artificial Sequence
  Synthetic Oligonucleotide Sequence
ggctcatcgatgacccaagatggcggcgcgttggctaatcccggtctaagtagtgacatgttt

SEQ ID NO: 244 - DNA, 36 bp, Artificial Sequence
  Synthetic Oligonucleotide Sequence
tcaccatgtaccaacggtctaagtagtgacatgttt

SEQ ID NO: 245 - DNA, 43 bp, Artificial Sequence
  Synthetic Oligonucleotide Sequence
ggctcatcgatgacccaagatggcggctcaccatgtaccaacg

SEQ ID NO: 246 - DNA, 63 bp, Artificial Sequence
  Synthetic Oligonucleotide Sequence
ggctcatcgatgacccaagatggcggctcaccatgtaccaacggtctaagtagtgacatgttt

SEQ ID NO: 247 - DNA, 38 bp, Artificial Sequence
  Synthetic Oligonucleotide Sequence
tatgaatgcgacccggaagtctaagtagtgacatgttt

SEQ ID NO: 248 - DNA, 45 bp, Artificial Sequence
  Synthetic Oligonucleotide Sequence
ggctcatcgatgacccaagatggcggctatgaatgcgacccggaa

SEQ ID NO: 249 - DNA, 65 bp, Artificial Sequence
  Synthetic Oligonucleotide Sequence
ggctcatcgatgacccaagatggcggctatgaatgcgacccggaagtctaagtagtgacatgttt

SEQ ID NO: 250 - DNA, 38 bp, Artificial Sequence
  Synthetic Oligonucleotide Sequence
aacaatggtcactgcatcgtctaagtagtgacatgttt

SEQ ID NO: 251 - DNA, 45 bp, Artificial Sequence
  Synthetic Oligonucleotide Sequence
ggctcatcgatgacccaagatggcggcaacaatggtcactgcatc

SEQ ID NO: 252 - DNA, 65 bp, Artificial Sequence
  Synthetic Oligonucleotide Sequence
ggctcatcgatgacccaagatggcggcaacaatggtcactgcatcgtctaagtagtgacatgttt

SEQ ID NO: 253 - DNA, 40 bp, Artificial Sequence
  Synthetic Oligonucleotide Sequence
gggccgtttcccggacataagtctaagtagtgacatgttt

SEQ ID NO: 254 - DNA, 47 bp, Artificial Sequence
  Synthetic Oligonucleotide Sequence
ggctcatcgatgacccaagatggcggcgggccgtttcccggacataa

SEQ ID NO: 255 - DNA, 67 bp, Artificial Sequence
  Synthetic Oligonucleotide Sequence
ggctcatcgatgacccaagatggcggcgggccgtttcccggacataagtctaagtagtgacatgttt

SEQ ID NO: 256 - DNA, 40 bp, Artificial Sequence
  Synthetic Oligonucleotide Sequence
aggttgagtccgcatctgaagtctaagtagtgacatgttt

SEQ ID NO: 257 - DNA, 47 bp, Artificial Sequence
  Synthetic Oligonucleotide Sequence
ggctcatcgatgacccaagatggcggcaggttgagtccgcatctgaa

SEQ ID NO: 258 - DNA, 67 bp, Artificial Sequence
  Synthetic Oligonucleotide Sequence
ggctcatcgatgacccaagatggcggcaggttgagtccgcatctgaagtctaagtagtgacatgttt

SEQ ID NO: 259 - DNA, 42 bp, Artificial Sequence
  Synthetic Oligonucleotide Sequence
tcgaccaagagccgctagatgcgtctaagtagtgacatgttt

SEQ ID NO: 260 - DNA, 49 bp, Artificial Sequence
  Synthetic Oligonucleotide Sequence
ggctcatcgatgacccaagatggcggctcgaccaagagccgctagatgc

SEQ ID NO: 261 - DNA, 69 bp, Artificial Sequence
  Synthetic Oligonucleotide Sequence
ggctcatcgatgacccaagatggcggctcgaccaagagccgctagatgcgtctaagtagtgacatgttt

SEQ ID NO: 262 - DNA, 42 bp, Artificial Sequence
  Synthetic Oligonucleotide Sequence
agctcgtgtcaagccgtcgcctgtctaagtagtgacatgttt

SEQ ID NO: 263 - DNA, 49 bp, Artificial Sequence
  Synthetic Oligonucleotide Sequence
ggctcatcgatgacccaagatggcggcagctcgtgtcaagccgtcgcct

SEQ ID NO: 264 - DNA, 69 bp, Artificial Sequence
  Synthetic Oligonucleotide Sequence
ggctcatcgatgacccaagatggcggcagctcgtgtcaagccgtcgcctgtctaagtagtgacatgttt

SEQ ID NO: 265 - DNA, 44 bp, Artificial Sequence
  Synthetic Oligonucleotide Sequence
tgaaagagttgtcagtttgctggtgtctaagtagtgacatgttt

SEQ ID NO: 266 - DNA, 51 bp, Artificial Sequence
  Synthetic Oligonucleotide Sequence
ggctcatcgatgacccaagatggcggctgaaagagttgtcagtttgctggt

SEQ ID NO: 267 - DNA, 71 bp, Artificial Sequence
  Synthetic Oligonucleotide Sequence
ggctcatcgatgacccaagatggcggctgaaagagttgtcagtttgctggtgtctaagtagtgacatgttt

SEQ ID NO: 268 - DNA, 45 bp, Artificial Sequence
  Synthetic Oligonucleotide Sequence
tcaggtaaaggttcctcacgctaccgtctaagtagtgacatgttt

SEQ ID NO: 269 - DNA, 52 bp, Artificial Sequence
  Synthetic Oligonucleotide Sequence
ggctcatcgatgacccaagatggcggctcaggtaaaggttcctcacgctacc

SEQ ID NO: 270 - DNA, 72 bp, Artificial Sequence
  Synthetic Oligonucleotide Sequence
ggctcatcgatgacccaagatggcggctcaggtaaaggttcctcacgctaccgtctaagtagtgacatgttt

SEQ ID NO: 271 - DNA, 27 bp, Artificial Sequence
  Synthetic Oligonucleotide Sequence
ggctcatcgatgacccaagatggcggc

SEQ ID NO: 272 - DNA, 47 bp, Artificial Sequence
  Synthetic Oligonucleotide Sequence
gtcatatgcgacgatctcagggctcatcgatgacccaagatggcggc

SEQ ID NO: 273 - DNA, 57 bp, Artificial Sequence
  Synthetic Oligonucleotide Sequence
gtccccatcggagggcatcttatcgtgcctggctcatcgatgacccaagatggcggc

SEQ ID NO: 274 - DNA, 57 bp, Artificial Sequence
  Synthetic Oligonucleotide Sequence
ccgccctccttcgccccccggtgaaataacggctcatcgatgacccaagatggcggc

SEQ ID NO: 275 - DNA, 57 bp, Artificial Sequence
  Synthetic Oligonucleotide Sequence
aatgctcacctctattcgggacttgagtacggctcatcgatgacccaagatggcggc

SEQ ID NO: 276 - DNA, 57 bp, Artificial Sequence
  Synthetic Oligonucleotide Sequence
gtcggaacgccaggtacagttagcgcatccggctcatcgatgacccaagatggcggc

SEQ ID NO: 277 - DNA, 57 bp, Artificial Sequence
  Synthetic Oligonucleotide Sequence
gtgatgctttatgagattccggtctccgacggctcatcgatgacccaagatggcggc

SEQ ID NO: 278 - DNA, 57 bp, Artificial Sequence
  Synthetic Oligonucleotide Sequence
gacggtgcatcacccgcatttgctgtagcgggctcatcgatgacccaagatggcggc

SEQ ID NO: 279 - DNA, 57 bp, Artificial Sequence
  Synthetic Oligonucleotide Sequence
aagccaaaattacaatcgatccctaccaacggctcatcgatgacccaagatggcggc

SEQ ID NO: 280 - DNA, 57 bp, Artificial Sequence
  Synthetic Oligonucleotide Sequence
atcttgcaccttcccagatgtaaaccccctggctcatcgatgacccaagatggcggc

SEQ ID NO: 281 - DNA, 57 bp, Artificial Sequence
  Synthetic Oligonucleotide Sequence
cggagaataccctcgactgtatcatatcgtggctcatcgatgacccaagatggcggc

SEQ ID NO: 282 - DNA, 57 bp, Artificial Sequence
  Synthetic Oligonucleotide Sequence
ttcatcgaggtacattggtgctattccattggctcatcgatgacccaagatggcggc

SEQ ID NO: 283 - DNA, 57 bp, Artificial Sequence
  Synthetic Oligonucleotide Sequence
aggagaaccagcctggagcgtttaagcatcggctcatcgatgacccaagatggcggc

SEQ ID NO: 284 - DNA, 57 bp, Artificial Sequence
  Synthetic Oligonucleotide Sequence
gatgtcctaaaatgaggcgtggcaatagagggctcatcgatgacccaagatggcggc

SEQ ID NO: 285 - DNA, 57 bp, Artificial Sequence
  Synthetic Oligonucleotide Sequence
cagagtcatgtatacccactgtcggtcgaaggctcatcgatgacccaagatggcggc

SEQ ID NO: 286 - DNA, 57 bp, Artificial Sequence
  Synthetic Oligonucleotide Sequence
gtcaggctagggggttatcccagcaacggcggctcatcgatgacccaagatggcggc

SEQ ID NO: 287 - DNA, 57 bp, Artificial Sequence
  Synthetic Oligonucleotide Sequence
tttttgacagtgatgaagagggaggtacgaggctcatcgatgacccaagatggcggc

SEQ ID NO: 288 - DNA, 57 bp, Artificial Sequence
  Synthetic Oligonucleotide Sequence
ctatggttcgttactgaatcgaaaagccgcggctcatcgatgacccaagatggcggc

SEQ ID NO: 289 - DNA, 57 bp, Artificial Sequence
  Synthetic Oligonucleotide Sequence
tagctatcaaaacaggcgtcatcggttaagggctcatcgatgacccaagatggcggc

SEQ ID NO: 290 - DNA, 57 bp, Artificial Sequence
  Synthetic Oligonucleotide Sequence
cctgcttagggtcacttaaactactggcgcggctcatcgatgacccaagatggcggc

SEQ ID NO: 291 - DNA, 57 bp, Artificial Sequence
  Synthetic Oligonucleotide Sequence
ggtgatggcccataccgatcacgcccgcagggctcatcgatgacccaagatggcggc

SEQ ID NO: 292 - DNA, 57 bp, Artificial Sequence
  Synthetic Oligonucleotide Sequence
cggcaggagggactgcgatttccatagagcggctcatcgatgacccaagatggcggc

SEQ ID NO: 293 - DNA, 57 bp, Artificial Sequence
  Synthetic Oligonucleotide Sequence
tggccggagagaggataggaagcgggactaggctcatcgatgacccaagatggcggc

SEQ ID NO: 294 - DNA, 57 bp, Artificial Sequence
  Synthetic Oligonucleotide Sequence
acacatcccaggactgccgtggcctacgtaggctcatcgatgacccaagatggcggc

SEQ ID NO: 295 - DNA, 57 bp, Artificial Sequence
  Synthetic Oligonucleotide Sequence
gacgagcttgttccaattcctcgagccgagggctcatcgatgacccaagatggcggc

SEQ ID NO: 296 - DNA, 57 bp, Artificial Sequence
  Synthetic Oligonucleotide Sequence
gttggggaggggcactacgacttagggctaggctcatcgatgacccaagatggcggc

SEQ ID NO: 297 - DNA, 57 bp, Artificial Sequence
  Synthetic Oligonucleotide Sequence
ggccgtcaatgtgttttgcacccaaccggaggctcatcgatgacccaagatggcggc

SEQ ID NO: 298 - DNA, 57 bp, Artificial Sequence
  Synthetic Oligonucleotide Sequence
tcccacgtccttcgacgcacactgtaacttggctcatcgatgacccaagatggcggc

SEQ ID NO: 299 - DNA, 52 bp, Artificial Sequence
  Synthetic Oligonucleotide Sequence
tcatgtatcgcccgtgggtaagctcggctcatcgatgacccaagatggcggc

SEQ ID NO: 300 - DNA, 52 bp, Artificial Sequence
  Synthetic Oligonucleotide Sequence
atgttatggagagtgggttaggcaaggctcatcgatgacccaagatggcggc

SEQ ID NO: 301 - DNA, 52 bp, Artificial Sequence
  Synthetic Oligonucleotide Sequence
atgagggagtaaggagattaggttcggctcatcgatgacccaagatggcggc

SEQ ID NO: 302 - DNA, 52 bp, Artificial Sequence
  Synthetic Oligonucleotide Sequence
gcccagcagttatacaattcgtggcggctcatcgatgacccaagatggcggc

SEQ ID NO: 303 - DNA, 52 bp, Artificial Sequence
  Synthetic Oligonucleotide Sequence
ttgggctctccagtagccgaacaaaggctcatcgatgacccaagatggcggc

SEQ ID NO: 304 - DNA, 52 bp, Artificial Sequence
  Synthetic Oligonucleotide Sequence
gtggttgctacagcctagcctagatggctcatcgatgacccaagatggcggc

SEQ ID NO: 305 - DNA, 52 bp, Artificial Sequence
  Synthetic Oligonucleotide Sequence
aggaggaaccggaagatctaatctgggctcatcgatgacccaagatggcggc

SEQ ID NO: 306 - DNA, 52 bp, Artificial Sequence
  Synthetic Oligonucleotide Sequence
gcgactgtggcaaccccatttcgcaggctcatcgatgacccaagatggcggc

SEQ ID NO: 307 - DNA, 52 bp, Artificial Sequence
  Synthetic Oligonucleotide Sequence
agttggatggatatctcgctcgtgaggctcatcgatgacccaagatggcggc

SEQ ID NO: 308 - DNA, 52 bp, Artificial Sequence
  Synthetic Oligonucleotide Sequence
cgctgtcctctctgacactaaaggtggctcatcgatgacccaagatggcggc

SEQ ID NO: 309 - DNA, 52 bp, Artificial Sequence
  Synthetic Oligonucleotide Sequence
atttcaatagtcaacccggtatccaggctcatcgatgacccaagatggcggc

SEQ ID NO: 310 - DNA, 52 bp, Artificial Sequence
  Synthetic Oligonucleotide Sequence
ggttggggggctcggctcatgtatcggctcatcgatgacccaagatggcggc

SEQ ID NO: 311 - DNA, 52 bp, Artificial Sequence
  Synthetic Oligonucleotide Sequence
taaggagactaggttccaatagctgggctcatcgatgacccaagatggcggc

SEQ ID NO: 312 - DNA, 52 bp, Artificial Sequence
  Synthetic Oligonucleotide Sequence
ttacacaaatcgtgggttggcctctggctcatcgatgacccaagatggcggc

SEQ ID NO: 313 - DNA, 52 bp, Artificial Sequence
  Synthetic Oligonucleotide Sequence
cgaaagcgttccgcaggacccccttggctcatcgatgacccaagatggcggc

SEQ ID NO: 314 - DNA, 52 bp, Artificial Sequence
  Synthetic Oligonucleotide Sequence
aaagtctgagaatgagtgataccatggctcatcgatgacccaagatggcggc

SEQ ID NO: 315 - DNA, 52 bp, Artificial Sequence
  Synthetic Oligonucleotide Sequence
atattggtagttttgtccgctgtagggctcatcgatgacccaagatggcggc

SEQ ID NO: 316 - DNA, 52 bp, Artificial Sequence
  Synthetic Oligonucleotide Sequence
cggaagatctaatctgcacgcaattggctcatcgatgacccaagatggcggc

SEQ ID NO: 317 - DNA, 57 bp, Artificial Sequence
  Synthetic Oligonucleotide Sequence
gcgcctcgttgggcagaagtttgtggaaatggctcatcgatgacccaagatggcggc

SEQ ID NO: 318 - DNA, 57 bp, Artificial Sequence
  Synthetic Oligonucleotide Sequence
atcttcacctaccgagttctacgggcctacggctcatcgatgacccaagatggcggc

SEQ ID NO: 319 - DNA, 57 bp, Artificial Sequence
  Synthetic Oligonucleotide Sequence
cccacaacttgcacccgctatgcgaccctgggctcatcgatgacccaagatggcggc

SEQ ID NO: 320 - DNA, 57 bp, Artificial Sequence
  Synthetic Oligonucleotide Sequence
gattagtggcccaacgggaacaaacttcctggctcatcgatgacccaagatggcggc

SEQ ID NO: 321 - DNA, 57 bp, Artificial Sequence
  Synthetic Oligonucleotide Sequence
cgcccgtcccagacccttactcactatggaggctcatcgatgacccaagatggcggc

SEQ ID NO: 322 - DNA, 57 bp, Artificial Sequence
  Synthetic Oligonucleotide Sequence
gagattgtaccctacagtccgattaccgatggctcatcgatgacccaagatggcggc

SEQ ID NO: 323 - DNA, 57 bp, Artificial Sequence
  Synthetic Oligonucleotide Sequence
cgcagtaaaagggcacaggtaattaccttaggctcatcgatgacccaagatggcggc

SEQ ID NO: 324 - DNA, 57 bp, Artificial Sequence
  Synthetic Oligonucleotide Sequence
agggtgtcttgaactactggcgcagcccatggctcatcgatgacccaagatggcggc

SEQ ID NO: 325 - DNA, 57 bp, Artificial Sequence
  Synthetic Oligonucleotide Sequence
tcggcggcgggtagtcagttcgctacctggggctcatcgatgacccaagatggcggc

SEQ ID NO: 326 - DNA, 57 bp, Artificial Sequence
  Synthetic Oligonucleotide Sequence
gatgtgatctggaccctacgggaggggacaggctcatcgatgacccaagatggcggc

SEQ ID NO: 327 - DNA, 57 bp, Artificial Sequence
  Synthetic Oligonucleotide Sequence
agtcccagatatgagagaagcgaagcataaggctcatcgatgacccaagatggcggc

SEQ ID NO: 328 - DNA, 52 bp, Artificial Sequence
  Synthetic Oligonucleotide Sequence
actattacaccacgtaccgtaggtcggctcatcgatgacccaagatggcggc

SEQ ID NO: 329 - DNA, 47 bp, Artificial Sequence; identical to SEQ ID NO: 272
  Synthetic Oligonucleotide Sequence

SEQ ID NO: 330 - DNA, 47 bp, Artificial Sequence
  Synthetic Oligonucleotide Sequence
tctccctatagtgagtcgtattaaattgtcatatgcgacgatctcag

SEQ ID NO: 331 - DNA, 74 bp, Artificial Sequence
  Synthetic Oligonucleotide Sequence
tctccctatagtgagtcgtattaaattgtcatatgcgacgatctcagggctcatcgatgacccaagatggcggc

SEQ ID NO: 332 - DNA, 57 bp, Artificial Sequence; identical to SEQ ID NO: 277
  Synthetic Oligonucleotide Sequence

SEQ ID NO: 333 - DNA, 57 bp, Artificial Sequence
  Synthetic Oligonucleotide Sequence
tctccctatagtgagtcgtattaaattgtgatgctttatgagattccggtctccgac

SEQ ID NO: 334 - DNA, 84 bp, Artificial Sequence
  Synthetic Oligonucleotide Sequence
tctccctatagtgagtcgtattaaattgtgatgctttatgagattccggtctccgacggctcatcgatgacccaagatggcggc

SEQ ID NO: 335 - DNA, 57 bp, Artificial Sequence; identical to SEQ ID NO: 282
  Synthetic Oligonucleotide Sequence

SEQ ID NO: 336 - DNA, 57 bp, Artificial Sequence
  Synthetic Oligonucleotide Sequence
tctccctatagtgagtcgtattaaattttcatcgaggtacattggtgctattccatt

SEQ ID NO: 337 - DNA, 84 bp, Artificial Sequence
  Synthetic Oligonucleotide Sequence
tctccctatagtgagtcgtattaaattttcatcgaggtacattggtgctattccattggctcatcgatgacccaagatggcggc

SEQ ID NO: 338 - DNA, 57 bp, Artificial Sequence; identical to SEQ ID NO: 284
  Synthetic Oligonucleotide Sequence

SEQ ID NO: 339 - DNA, 57 bp, Artificial Sequence
  Synthetic Oligonucleotide Sequence
tctccctatagtgagtcgtattaaattgatgtcctaaaatgaggcgtggcaatagag

SEQ ID NO: 340 - DNA, 84 bp, Artificial Sequence
  Synthetic Oligonucleotide Sequence
tctccctatagtgagtcgtattaaattgatgtcctaaaatgaggcgtggcaatagagggctcatcgatgacccaagatggcggc

SEQ ID NO: 341 - DNA, 57 bp, Artificial Sequence; identical to SEQ ID NO: 285
  Synthetic Oligonucleotide Sequence

SEQ ID NO: 342 - DNA, 57 bp, Artificial Sequence
  Synthetic Oligonucleotide Sequence
tctccctatagtgagtcgtattaaattcagagtcatgtatacccactgtcggtcgaa

SEQ ID NO: 343 - DNA, 84 bp, Artificial Sequence
  Synthetic Oligonucleotide Sequence
tctccctatagtgagtcgtattaaattcagagtcatgtatacccactgtcggtcgaaggctcatcgatgacccaagatggcggc

SEQ ID NO: 344 - DNA, 52 bp, Artificial Sequence; identical to SEQ ID NO: 300
  Synthetic Oligonucleotide Sequence

SEQ ID NO: 345 - DNA, 52 bp, Artificial Sequence
  Synthetic Oligonucleotide Sequence
tctccctatagtgagtcgtattaaattatgttatggagagtgggttaggcaa

SEQ ID NO: 346 - DNA, 79 bp, Artificial Sequence
  Synthetic Oligonucleotide Sequence
tctccctatagtgagtcgtattaaattatgttatggagagtgggttaggcaaggctcatcgatgacccaagatggcggc

SEQ ID NO: 347 - DNA, 52 bp, Artificial Sequence; identical to SEQ ID NO: 314
  Synthetic Oligonucleotide Sequence

SEQ ID NO: 348 - DNA, 52 bp, Artificial Sequence
  Synthetic Oligonucleotide Sequence
tctccctatagtgagtcgtattaaattaaagtctgagaatgagtgataccat

SEQ ID NO: 349 - DNA, 79 bp, Artificial Sequence
  Synthetic Oligonucleotide Sequence
tctccctatagtgagtcgtattaaattaaagtctgagaatgagtgataccatggctcatcgatgacccaagatggcggc

SEQ ID NO: 350 - DNA, 57 bp, Artificial Sequence; identical to SEQ ID NO: 319
  Synthetic Oligonucleotide Sequence

SEQ ID NO: 351 - DNA, 57 bp, Artificial Sequence
  Synthetic Oligonucleotide Sequence
tctccctatagtgagtcgtattaaattcccacaacttgcacccgctatgcgaccctg

SEQ ID NO: 352 - DNA, 84 bp, Artificial Sequence
  Synthetic Oligonucleotide Sequence
tctccctatagtgagtcgtattaaattcccacaacttgcacccgctatgcgaccctgggctcatcgatgacccaagatggcggc

SEQ ID NO: 353 - DNA, 57 bp, Artificial Sequence; identical to SEQ ID NO: 320
  Synthetic Oligonucleotide Sequence

SEQ ID NO: 354 - DNA, 57 bp, Artificial Sequence
  Synthetic Oligonucleotide Sequence
tctccctatagtgagtcgtattaaattgattagtggcccaacgggaacaaacttcct

SEQ ID NO: 355 - DNA, 84 bp, Artificial Sequence
  Synthetic Oligonucleotide Sequence
tctccctatagtgagtcgtattaaattgattagtggcccaacgggaacaaacttcctggctcatcgatgacccaagatggcggc

SEQ ID NO: 356 - DNA, 57 bp, Artificial Sequence; identical to SEQ ID NO: 321
  Synthetic Oligonucleotide Sequence

SEQ ID NO: 357 - DNA, 57 bp, Artificial Sequence
  Synthetic Oligonucleotide Sequence
tctccctatagtgagtcgtattaaattcgcccgtcccagacccttactcactatgga

SEQ ID NO: 358 - DNA, 84 bp, Artificial Sequence
  Synthetic Oligonucleotide Sequence
tctccctatagtgagtcgtattaaattcgcccgtcccagacccttactcactatggaggctcatcgatgacccaagatggcggc

SEQ ID NO: 359 - DNA, 24 bp, Artificial Sequence
  Synthetic Oligonucleotide Sequence
gaugcagugggcagcugugaggac

SEQ ID NO: 360 - DNA, 24 bp, Artificial Sequence
  Synthetic Oligonucleotide Sequence
ugugucuucaggaugaaacacaca

SEQ ID NO: 361 - DNA, 26 bp, Artificial Sequence
  Synthetic Oligonucleotide Sequence
aucuguuuuccugcccauccuuuaag

SEQ ID NO: 362 - DNA, 57 bp, Artificial Sequence
  Synthetic Oligonucleotide Sequence
aucuguuuuccugcccauccuuuaagtttaaaaaaaaaaaaaaaaaaaaaaaaaaaa

SEQ ID NO: 363 - DNA, 31 bp, Artificial Sequence
  Synthetic Oligonucleotide Sequence
ccactgcatcaggaacaaaagcgtgatcttg

SEQ ID NO: 364 - DNA, 43 bp, Artificial Sequence
  Synthetic Oligonucleotide Sequence
tggctaatcccgccactgcatcaggaacaaaagcgtgatcttg

SEQ ID NO: 365 - DNA, 39 bp, Artificial Sequence; identical to SEQ ID NO: 206
  Synthetic Oligonucleotide Sequence

SEQ ID NO: 366 - DNA, 70 bp, Artificial Sequence
  Synthetic Oligonucleotide Sequence
ggctcatcgatgacccaagatggcggctggctaatcccgccactgcatcaggaacaaaagcgtgatcttg

SEQ ID NO: 367 - DNA, 51 bp, Artificial Sequence
  Synthetic Oligonucleotide Sequence
aggttgagtccgcatctgaaccactgcatcaggaacaaaagcgtgatcttg

SEQ ID NO: 368 - DNA, 47 bp, Artificial Sequence; identical to SEQ ID NO: 257
  Synthetic Oligonucleotide Sequence

SEQ ID NO: 369 - DNA, 78 bp, Artificial Sequence
  Synthetic Oligonucleotide Sequence
ggctcatcgatgacccaagatggcggcaggttgagtccgcatctgaaccactgcatcaggaacaaaagcgtgatcttg

SEQ ID NO: 370 - DNA, 43 bp, Artificial Sequence
  Synthetic Oligonucleotide Sequence
atgtgcgcacaaccactgcatcaggaacaaaagcgtgatcttg

SEQ ID NO: 371 - DNA, 39 bp, Artificial Sequence; identical to SEQ ID NO: 224
  Synthetic Oligonucleotide Sequence

SEQ ID NO: 372 - DNA, 70 bp, Artificial Sequence
  Synthetic Oligonucleotide Sequence
ggctcatcgatgacccaagatggcggcatgtgcgcacaaccactgcatcaggaacaaaagcgtgatcttg

SEQ ID NO: 373 - DNA, 49 bp, Artificial Sequence
  Synthetic Oligonucleotide Sequence
tatgaatgcgacccggaaccactgcatcaggaacaaaagcgtgatcttg

SEQ ID NO: 374 - DNA, 45 bp, Artificial Sequence; identical to SEQ ID NO: 248
  Synthetic Oligonucleotide Sequence

SEQ ID NO: 375 - DNA, 76 bp, Artificial Sequence
  Synthetic Oligonucleotide Sequence
ggctcatcgatgacccaagatggcggctatgaatgcgacccggaaccactgcatcaggaacaaaagcgtgatcttg

SEQ ID NO: 376 - DNA, 43 bp, Artificial Sequence
  Synthetic Oligonucleotide Sequence
catgtaccaacgccactgcatcaggaacaaaagcgtgatcttg

SEQ ID NO: 377 - DNA, 39 bp, Artificial Sequence; identical to SEQ ID NO: 212
  Synthetic Oligonucleotide Sequence

SEQ ID NO: 378 - DNA, 70 bp, Artificial Sequence
  Synthetic Oligonucleotide Sequence
ggctcatcgatgacccaagatggcggccatgtaccaacgccactgcatcaggaacaaaagcgtgatcttg

SEQ ID NO: 379 - DNA, 43 bp, Artificial Sequence
  Synthetic Oligonucleotide Sequence
aatctccgagcgccactgcatcaggaacaaaagcgtgatcttg

SEQ ID NO: 380 - DNA, 39 bp, Artificial Sequence; identical to SEQ ID NO: 230
  Synthetic Oligonucleotide Sequence

SEQ ID NO: 381 - DNA, 70 bp, Artificial Sequence
  Synthetic Oligonucleotide Sequence
ggctcatcgatgacccaagatggcggcaatctccgagcgccactgcatcaggaacaaaagcgtgatcttg

SEQ ID NO: 382 - DNA, 47 bp, Artificial Sequence
  Synthetic Oligonucleotide Sequence
tcaccatgtaccaacgccactgcatcaggaacaaaagcgtgatcttg

SEQ ID NO: 383 - DNA, 43 bp, Artificial Sequence; identical to SEQ ID NO: 245
  Synthetic Oligonucleotide Sequence

SEQ ID NO: 384 - DNA, 74 bp, Artificial Sequence
  Synthetic Oligonucleotide Sequence
ggctcatcgatgacccaagatggcggctcaccatgtaccaacgccactgcatcaggaacaaaagcgtgatcttg

SEQ ID NO: 385 - DNA, 49 bp, Artificial Sequence
  Synthetic Oligonucleotide Sequence
aacaatggtcactgcatcccactgcatcaggaacaaaagcgtgatcttg

SEQ ID NO: 386 - DNA, 45 bp, Artificial Sequence; identical to SEQ ID NO: 251
  Synthetic Oligonucleotide Sequence

SEQ ID NO: 387 - DNA, 76 bp, Artificial Sequence
  Synthetic Oligonucleotide Sequence
ggctcatcgatgacccaagatggcggcaacaatggtcactgcatcccactgcatcaggaacaaaagcgtgatcttg

SEQ ID NO: 388 - DNA, 51 bp, Artificial Sequence
  Synthetic Oligonucleotide Sequence
gggccgtttcccggacataaccactgcatcaggaacaaaagcgtgatcttg

SEQ ID NO: 389 - DNA, 47 bp, Artificial Sequence; identical to SEQ ID NO: 254
  Synthetic Oligonucleotide Sequence

SEQ ID NO: 390 - DNA, 78 bp, Artificial Sequence
  Synthetic Oligonucleotide Sequence
ggctcatcgatgacccaagatggcggcgggccgtttcccggacataaccactgcatcaggaacaaaagcgtgatcttg

SEQ ID NO: 391 - DNA, 55 bp, Artificial Sequence
  Synthetic Oligonucleotide Sequence
tgaaagagttgtcagtttgctggtccactgcatcaggaacaaaagcgtgatcttg

SEQ ID NO: 392 - DNA, 51 bp, Artificial Sequence; identical to SEQ ID NO: 266
  Synthetic Oligonucleotide Sequence

SEQ ID NO: 393 - DNA, 82 bp, Artificial Sequence
  Synthetic Oligonucleotide Sequence
ggctcatcgatgacccaagatggcggctgaaagagttgtcagtttgctggtccactgcatcaggaacaaaagcgtgatcttg

SEQ ID NO: 394 - DNA, 56 bp, Artificial Sequence
  Synthetic Oligonucleotide Sequence
tcaggtaaaggttcctcacgctaccccactgcatcaggaacaaaagcgtgatcttg

SEQ ID NO: 395 - DNA, 52 bp, Artificial Sequence; identical to SEQ ID NO: 269
  Synthetic Oligonucleotide Sequence

SEQ ID NO: 396 - DNA, 83 bp, Artificial Sequence
  Synthetic Oligonucleotide Sequence
ggctcatcgatgacccaagatggcggctcaggtaaaggttcctcacgctaccccactgcatcaggaacaaaagcgtgatcttg

SEQ ID NO: 397 - DNA, 22 bp, Artificial Sequence
  Synthetic Oligonucleotide Sequence
gctgtggctgacctgaaatacc

SEQ ID NO: 398 - DNA, 52 bp, Artificial Sequence
  Synthetic Oligonucleotide Sequence
gtgatgctttatgagattccggtctccgacgctgtggctgacctgaaatacc

SEQ ID NO: 399 - DNA, 52 bp, Artificial Sequence
  Synthetic Oligonucleotide Sequence
gatgtcctaaaatgaggcgtggcaatagaggctgtggctgacctgaaatacc

SEQ ID NO: 400 - DNA, 52 bp, Artificial Sequence
  Synthetic Oligonucleotide Sequence
cagagtcatgtatacccactgtcggtcgaagctgtggctgacctgaaatacc

SEQ ID NO: 401 - DNA, 47 bp, Artificial Sequence
  Synthetic Oligonucleotide Sequence
atgttatggagagtgggttaggcaagctgtggctgacctgaaatacc

SEQ ID NO: 402 - DNA, 47 bp, Artificial Sequence
  Synthetic Oligonucleotide Sequence
aaagtctgagaatgagtgataccatgctgtggctgacctgaaatacc

SEQ ID NO: 403 - DNA, 52 bp, Artificial Sequence
  Synthetic Oligonucleotide Sequence
cccacaacttgcacccgctatgcgaccctggctgtggctgacctgaaatacc

SEQ ID NO: 404 - DNA, 52 bp, Artificial Sequence
  Synthetic Oligonucleotide Sequence
gattagtggcccaacgggaacaaacttcctgctgtggctgacctgaaatacc

SEQ ID NO: 405 - DNA, 52 bp, Artificial Sequence
  Synthetic Oligonucleotide Sequence
cgcccgtcccagacccttactcactatggagctgtggctgacctgaaatacc

SEQ ID NO: 406 - DNA, 24 bp, Artificial Sequence
  Synthetic Oligonucleotide Sequence
gaugcagugggcagcugugaggac

SEQ ID NO: 407 - DNA, 24 bp, Artificial Sequence
  Synthetic Oligonucleotide Sequence
ugugucuucaggaugaaacacaca

SEQ ID NO: 408 - DNA, 26 bp, Artificial Sequence
  Synthetic Oligonucleotide Sequence
cgaacuugcgcacacacgucauugga

SEQ ID NO: 409 - DNA, 59 bp, Artificial Sequence
  Synthetic Oligonucleotide Sequence
cgaacuugcgcacacacgucauuggatttaaaaaaaaaaaaaaaaaaaaaaaaaaaaaa